European Patent Specification EP 3 359 573 B1, published January 4, 2023. Title: LABELING OF ANTIBODIES. Applicant: WHITEHEAD INSTITUTE FOR BIOMEDICAL RESEARCH THE GENERAL HOSPITAL CORPORATION D/B/A MASSACHUSETTS GENERAL HOSPITAL. Application Not Yet Assigned. The sequence listing filed with the application follows.

SEQUENCE LISTING (81 sequences)

SEQ ID NO: 1 - DNA, 378 bp, Artificial Sequence
  Synthetic Polynucleotide
caggtgcagctgcaggagtcagggggaggattggtgcagcctggggggtctctgagactctcctgtacagcctctggattcacattcagtacttactacatgagctgggtccgcaaggctccagggaaggggcccgagtgggtctcagttatgaatagtagtggtggtgacacaaggtatgcagacttcgtgaagggccgattcaccatctccagagacaacgccaagaacacactgtatctccaaatgaacagcctgaaacctgaggatacggccctgtattactgtgcgcaaggtagatcagatatatacccaaccttcacgcggggccaggggacccaggtcaccgtctcctcaggaggactgccggaaaccggc

SEQ ID NO: 2 - protein, 133 aa, Artificial Sequence
  Synthetic Polypeptide
QVQLQESGGGLVQPGGSLRLSCTASGFTFSTYYMSWVRKAPGKGPEWVSVMNSSGGDTRYADFVKGRFTISRDNAKNTLYLQMNSLKPEDTALYYCAQGRSDIYPTFTRGQGTQVTVSSGSLPETGGHHHHHH

SEQ ID NO: 3 - DNA, 411 bp, Artificial Sequence
  Synthetic Polynucleotide
caggttcaactgcaagagagtggcgggggcctggttcagaccggtggttctctccggctctcgtgtgccgcaagtggagtagattttaactggtatagcatgggttggttcaggcaagcccctggcaaagagcgggagtatgtggcttcgattgaccagggaggcgagttggattacgcaatatcagtaaagggcagattcacgatctcccgagacaacgcgaagaatatggtgtatctccagatgaattcgttaaagcccgaagacaccgctgtatactactgtgccgcagatttttccggccggggtgcgtcaaaccctgacaagtataaatattggggacagggaacccaagtgaccgtcagcagcggtgggttgcccgaaactggaggacaccatcaccatcaccat

SEQ ID NO: 4 - protein, 137 aa, Artificial Sequence
  Synthetic Polypeptide
QVQLQESGGGLVQTGGSLRLSCAASGVDFNWYSMGWFRQAPGKEREYVASIDQGGELDYAISVKGRFTISRDNAKNMVYLQMNSLKPEDTAVYYCAADFSGRGASNPDKYKYWGQGTQVTVSSGGLPETGGHHHHHH

SEQ ID NO: 5 - protein, 12 aa, Artificial Sequence
  Synthetic Polypeptide
LPETGGHHHHHH

SEQ ID NO: 6 - protein, 8 aa, Artificial Sequence
  Synthetic Polypeptide
GGHHHHHH

SEQ ID NO: 7 - protein, 4 aa, Artificial Sequence
  Synthetic Polypeptide
LPET

SEQ ID NO: 8 - protein, 7 aa, Artificial Sequence
  Synthetic Polypeptide
LPETGGG

SEQ ID NO: 9 - protein, 7 aa, Artificial Sequence
  Synthetic Polypeptide
  misc_feature (6)..(7): Xaa can be any naturally occurring amino acid
LPETGXX

SEQ ID NO: 10 - protein, 8 aa, Artificial Sequence
  Synthetic Polypeptide
LPETGGGC

SEQ ID NO: 11 - protein, 5 aa, Artificial Sequence
  Synthetic Polypeptide
LPETG

SEQ ID NO: 12 - protein, 4 aa, Artificial Sequence
  Synthetic Polypeptide
GGGC

SEQ ID NO: 13 - protein, 6 aa, Artificial Sequence
  Synthetic Polypeptide
  misc_feature (3)..(3): Xaa can be any naturally occurring amino acid
  misc_feature (6)..(6): Xaa can be any naturally occurring amino acid
LPXTGX

SEQ ID NO: 14 - protein, 7 aa, Artificial Sequence
  Synthetic Polypeptide
  misc_feature (3)..(3): Xaa can be any naturally occurring amino acid
LPXTGGG

SEQ ID NO: 15 - protein, 5 aa, Artificial Sequence
  Synthetic Polypeptide
  misc_feature (3)..(3): Xaa can be any naturally occurring amino acid
  misc_feature (5)..(5): Xaa can be any naturally occurring amino acid
LPXTX

SEQ ID NO: 16 - protein, 5 aa, Artificial Sequence
  Synthetic Polypeptide
  misc_feature (3)..(3): Xaa can be any naturally occurring amino acid
  misc_feature (5)..(5): Xaa can be any naturally occurring amino acid
NPXTX

SEQ ID NO: 17 - protein, 5 aa, Artificial Sequence
  Synthetic Polypeptide
  misc_feature (3)..(3): Xaa can be any naturally occurring amino acid
LPXAG

SEQ ID NO: 18 - protein, 5 aa, Artificial Sequence
  Synthetic Polypeptide
LPETA

SEQ ID NO: 19 - protein, 5 aa, Artificial Sequence
  Synthetic Polypeptide
NPQTN

SEQ ID NO: 20 - protein, 5 aa, Artificial Sequence
  Synthetic Polypeptide
NPKTG

SEQ ID NO: 21 - protein, 5 aa, Artificial Sequence
  Synthetic Polypeptide
LPSTG

SEQ ID NO: 22 - protein, 4 aa, Artificial Sequence
  Synthetic Polypeptide
  misc_feature (3)..(3): Xaa can be any naturally occurring amino acid
LPXT

SEQ ID NO: 23 - protein, 5 aa, Artificial Sequence
  Synthetic Polypeptide
LPKTG

SEQ ID NO: 24 - protein, 5 aa, Artificial Sequence
  Synthetic Polypeptide
LPATG

SEQ ID NO: 25 - protein, 5 aa, Artificial Sequence
  Synthetic Polypeptide
LPNTG

SEQ ID NO: 26 - protein, 5 aa, Artificial Sequence
  Synthetic Polypeptide
LPNAG

SEQ ID NO: 27 - protein, 5 aa, Artificial Sequence
  Synthetic Polypeptide
  misc_feature (3)..(3): Xaa can be any naturally occurring amino acid
LPXTA

SEQ ID NO: 28 - protein, 5 aa, Artificial Sequence
  Synthetic Polypeptide
LPNTA

SEQ ID NO: 29 - protein, 5 aa, Artificial Sequence
  Synthetic Polypeptide
LPETA

SEQ ID NO: 30 - protein, 5 aa, Artificial Sequence
  Synthetic Polypeptide
  misc_feature (3)..(3): Xaa can be any naturally occurring amino acid
LGXTG

SEQ ID NO: 31 - protein, 5 aa, Artificial Sequence
  Synthetic Polypeptide
LGATG

SEQ ID NO: 32 - protein, 5 aa, Artificial Sequence
  Synthetic Polypeptide
  misc_feature (3)..(3): Xaa can be any naturally occurring amino acid
IPXTG

SEQ ID NO: 33 - protein, 5 aa, Artificial Sequence
  Synthetic Polypeptide
IPNTG

SEQ ID NO: 34 - protein, 5 aa, Artificial Sequence
  Synthetic Polypeptide
IPETG

SEQ ID NO: 35 - protein, 5 aa, Artificial Sequence
  Synthetic Polypeptide
  misc_feature (3)..(3): Xaa is Gln or Lys
  misc_feature (4)..(4): Xaa is Thr or absent
  misc_feature (5)..(5): Xaa is Asn, Gly, or absent
NPXXX

SEQ ID NO: 36 - protein, 5 aa, Artificial Sequence
  Synthetic Polypeptide
NPQTN

SEQ ID NO: 37 - protein, 5 aa, Artificial Sequence
  Synthetic Polypeptide
NPKTG

SEQ ID NO: 38 - protein, 5 aa, Artificial Sequence
  Synthetic Polypeptide
NSKTA

SEQ ID NO: 39 - protein, 5 aa, Artificial Sequence
  Synthetic Polypeptide
NPQTG

SEQ ID NO: 40 - protein, 5 aa, Artificial Sequence
  Synthetic Polypeptide
NAKTN

SEQ ID NO: 41 - protein, 5 aa, Artificial Sequence
  Synthetic Polypeptide
NPQSS

SEQ ID NO: 42 - protein, 5 aa, Artificial Sequence
  Synthetic Polypeptide
  misc_feature (3)..(3): Xaa is Glu, Ala, Ser, or His
NAXTG

SEQ ID NO: 43 - protein, 5 aa, Artificial Sequence
  Synthetic Polypeptide
  misc_feature (3)..(3): Xaa can be any naturally occurring amino acid
LPXTA

SEQ ID NO: 44 - protein, 5 aa, Artificial Sequence
  Synthetic Polypeptide
  misc_feature (3)..(3): Xaa can be any naturally occurring amino acid
LAXTG

SEQ ID NO: 45 - protein, 6 aa, Artificial Sequence
  Synthetic Polypeptide
QVPTGV

SEQ ID NO: 46 - protein, 5 aa, Artificial Sequence
  Synthetic Polypeptide
  misc_feature (3)..(3): Xaa can be any naturally occurring amino acid
TLXTC

SEQ ID NO: 47 - protein, 206 aa, S. aureus
MKKWTNRLMTIAGVVLILVAAYLFAKPHIDNYLHDKDKDEKIEQYDKNVKEQASKDNKQQAKPQIPKDKSKVAGYIEIPDADIKEPVYPGPATPEQLNRGVSFAEENESLDDQNISIAGHTFIDRPNYQFTNLKAAKKGSMVYFKVGNETRKYKMTSIRDVKPTDVEVLDEQKGKDKQLTLITCDDYNEKTGVWEKRKIFVATEVK

SEQ ID NO: 48 - protein, 206 aa, S. aureus
MKKWTNRLMTIAGVVLILVAAYLFAKPHIDNYLHDKDKDEKIEQYDKNVKEQASKDKKQQAKPQIPKDKSKVAGYIEIPDADIKEPVYPGPATPEQLNRGVSFAEENESLDDQNISIAGHTFIDRPNYQFTNLKAAKKGSMVYFKVGNETRKYKMTSIRDVKPTDVGVLDEQKGKDKQLTLITCDDYNEKTGVWEKRKIFVATEVK

SEQ ID NO: 49 - protein, 148 aa, Artificial Sequence
  Synthetic Polypeptide
MQAKPQIPKDKSKVAGYIEIPDADIKEPVYPGPATREQLNRGVSFAEENESLDDQNISIAGHTFIDRPNYQFTNLKAAKKGSMVYFKVGNETRKYKMTSIRNVKPTAVEVLDEQKGKDKQLTLITCDDYNEETGVWETRKIFVATEVK

SEQ ID NO: 50 - protein, 6 aa, Artificial Sequence
  Synthetic Polypeptide
  misc_feature (3)..(3): Xaa is Gln or Lys
  misc_feature (5)..(5): Xaa is Ala or Ser
LPXTXT

SEQ ID NO: 51 - protein, 5 aa, Artificial Sequence
  Synthetic Polypeptide
  misc_feature (3)..(3): Xaa can be any naturally occurring amino acid
  misc_feature (5)..(5): Xaa can be any naturally occurring amino acid
LPXTX

SEQ ID NO: 52 - protein, 5 aa, Artificial Sequence
  Synthetic Polypeptide
LPSTS

SEQ ID NO: 53 - protein, 5 aa, Artificial Sequence
  Synthetic Polypeptide
LPITG

SEQ ID NO: 54 - protein, 5 aa, Artificial Sequence
  Synthetic Polypeptide
LPDTA

SEQ ID NO: 55 - protein, 5 aa, Artificial Sequence
  Synthetic Polypeptide
SPKTG

SEQ ID NO: 56 - protein, 5 aa, Artificial Sequence
  Synthetic Polypeptide
LAETG

SEQ ID NO: 57 - protein, 5 aa, Artificial Sequence
  Synthetic Polypeptide
LAATG

SEQ ID NO: 58 - protein, 5 aa, Artificial Sequence
  Synthetic Polypeptide
LAHTG

SEQ ID NO: 59 - protein, 5 aa, Artificial Sequence
  Synthetic Polypeptide
LASTG

SEQ ID NO: 60 - protein, 5 aa, Artificial Sequence
  Synthetic Polypeptide
LPLTG

SEQ ID NO: 61 - protein, 5 aa, Artificial Sequence
  Synthetic Polypeptide
LSRTG

SEQ ID NO: 62 - protein, 5 aa, Artificial Sequence
  Synthetic Polypeptide
VPDTG

SEQ ID NO: 63 - protein, 5 aa, Artificial Sequence
  Synthetic Polypeptide
IPQTG

SEQ ID NO: 64 - protein, 5 aa, Artificial Sequence
  Synthetic Polypeptide
YPRRG

SEQ ID NO: 65 - protein, 5 aa, Artificial Sequence
  Synthetic Polypeptide
LPMTG

SEQ ID NO: 66 - protein, 5 aa, Artificial Sequence
  Synthetic Polypeptide
LAFTG

SEQ ID NO: 67 - protein, 5 aa, Artificial Sequence
  Synthetic Polypeptide
LPQTS

SEQ ID NO: 68 - protein, 4 aa, Artificial Sequence
  Synthetic Polypeptide
  misc_feature (3)..(3): Xaa can be any naturally occurring amino acid
LAXT

SEQ ID NO: 69 - protein, 4 aa, Artificial Sequence
  Synthetic Polypeptide
  misc_feature (3)..(3): Xaa can be any naturally occurring amino acid
LPXA

SEQ ID NO: 70 - protein, 4 aa, Artificial Sequence
  Synthetic Polypeptide
  misc_feature (3)..(3): Xaa can be any naturally occurring amino acid
LGXT

SEQ ID NO: 71 - protein, 4 aa, Artificial Sequence
  Synthetic Polypeptide
  misc_feature (3)..(3): Xaa can be any naturally occurring amino acid
IPXT

SEQ ID NO: 72 - protein, 4 aa, Artificial Sequence
  Synthetic Polypeptide
  misc_feature (3)..(3): Xaa can be any naturally occurring amino acid
NPXT

SEQ ID NO: 73 - protein, 4 aa, Artificial Sequence
  Synthetic Polypeptide
NPQS

SEQ ID NO: 74 - protein, 4 aa, Artificial Sequence
  Synthetic Polypeptide
LPST

SEQ ID NO: 75 - protein, 4 aa, Artificial Sequence
  Synthetic Polypeptide
NSKT

SEQ ID NO: 76 - protein, 4 aa, Artificial Sequence
  Synthetic Polypeptide
NPQT

SEQ ID NO: 77 - protein, 4 aa, Artificial Sequence
  Synthetic Polypeptide
NAKT

SEQ ID NO: 78 - protein, 4 aa, Artificial Sequence
  Synthetic Polypeptide
LPIT

SEQ ID NO: 79 - protein, 4 aa, Artificial Sequence
  Synthetic Polypeptide
LAET

SEQ ID NO: 80 - protein, 4 aa, Artificial Sequence
  Synthetic Polypeptide
NPQS

SEQ ID NO: 81 - protein, 5 aa, Artificial Sequence
  Synthetic Polypeptide
  misc_feature (3)..(3): Xaa can be any naturally occurring amino acid
LPXTG